European Patent Application EP 4 516 810 A2, published March 5, 2025. Title: Bispecific Anti-BCMA X Anti-CD3 Antibodies and Uses Thereof. Applicant: Regeneron Pharmaceuticals, Inc. Application EP. The sequence listing filed with the application follows.

SEQUENCE LISTING (125 sequences)

SEQ ID NO: 1 - DNA, 366 bp, synthetic construct
  misc_feature 1..366: note = synthetic
  source 1..366: mol_type = other DNA
caggtgcagctggtggagtcggggggaggcgtggtccagcctgggaggtccctgagactctcctgtgcagcctctggattcaccttcagtacctatggcattcactgggtccgccaggctccaggcaaggggctggagtgggtggcagttatattacatgatggaagtagtaactactatgcagagtccgtgaagggccgattcatcatctccagagacaattccaagaacacactgtatctgcaaatgaacagcctgagagctgaggacacggctctatattactgtacgaaaaggtattcagaagcagctggcccaaattggttcgacccctggggccagggaaccctggtcaccgtctcctca

SEQ ID NO: 2 - protein, 122 aa, synthetic construct
  REGION 1..122: note = synthetic
QVQLVESGGGVVQPGRSLRLSCAASGFTFSTYGIHWVRQAPGKGLEWVAVILHDGSSNYYAESVKGRFIISRDNSKNTLYLQMNSLRAEDTALYYCTKRYSEAAGPNWFDPWGQGTLVTVSS

SEQ ID NO: 3 - DNA, 24 bp, synthetic construct
  misc_feature 1..24: note = synthetic
  source 1..24: mol_type = other DNA
ggattcaccttcagtacctatggc

SEQ ID NO: 4 - protein, 8 aa, synthetic construct
  REGION 1..8: note = synthetic
GFTFSTYG

SEQ ID NO: 5 - DNA, 24 bp, synthetic construct
  misc_feature 1..24: note = synthetic
  source 1..24: mol_type = other DNA
atattacatgatggaagtagtaac

SEQ ID NO: 6 - protein, 8 aa, synthetic construct
  REGION 1..8: note = synthetic
ILHDGSSN

SEQ ID NO: 7 - DNA, 45 bp, synthetic construct
  misc_feature 1..45: note = synthetic
  source 1..45: mol_type = other DNA
acgaaaaggtattcagaagcagctggcccaaattggttcgacccc

SEQ ID NO: 8 - protein, 15 aa, synthetic construct
  REGION 1..15: note = synthetic
TKRYSEAAGPNWFDP

SEQ ID NO: 9 - DNA, 321 bp, synthetic construct
  misc_feature 1..321: note = synthetic
  source 1..321: mol_type = other DNA
gacatccagatgacccagtctccatcctccgtgtctgcatctgtaggagacagagtcaccatcacttgtcgggcgagtcggggaattagcagctggttagcctggtatcagcagaagccagggaaagcccctaagctcctgatccatgctgcatccagtttgcaaagtggggtcccatcaaggttcagcggcagtggatctgggacagatttcactctcaccatcagcagcctgcagcctgaagattttgctacttactattgtcaacaggctatcagtttcccattcactttcggccctgggaccaaagtggatatcaaa

SEQ ID NO: 10 - protein, 107 aa, synthetic construct
  REGION 1..107: note = synthetic
DIQMTQSPSSVSASVGDRVTITCRASRGISSWLAWYQQKPGKAPKLLIHAASSLQSGVPSRFSGSGSGTDFTLTISSLQPEDFATYYCQQAISFPFTFGPGTKVDIK

SEQ ID NO: 11 - DNA, 18 bp, synthetic construct
  misc_feature 1..18: note = synthetic
  source 1..18: mol_type = other DNA
cggggaattagcagctgg

SEQ ID NO: 12 - protein, 6 aa, synthetic construct
  REGION 1..6: note = synthetic
RGISSW

SEQ ID NO: 13-14 - skipped (2 entries)

SEQ ID NO: 15 - DNA, 27 bp, synthetic construct
  misc_feature 1..27: note = synthetic
  source 1..27: mol_type = other DNA
caacaggctatcagtttcccattcact

SEQ ID NO: 16 - protein, 9 aa, synthetic construct
  REGION 1..9: note = synthetic
QQAISFPFT

SEQ ID NO: 17 - DNA, 360 bp, synthetic construct
  misc_feature 1..360: note = synthetic
  source 1..360: mol_type = other DNA
gaggtgcagctggtggagtctgggggaggcttggtacagcctggggggtccctgagactctcctgtgcagcctctggattcacctttagcagctatgtcatgagttgggtccgccaggctccagggaagggactggagtgggtctcagctattattggtagtggtggtagcacatattacgcagactccgtgaagggccggttcaccatctccagagacaattccaagaacacgctgtatctgcaaatgaacagcctgagagccgaggacacggccgtatattactgtgcgaaaagagccggggataactggaactggttcgacccctggggccagggaaccctggtcaccgtctcctca

SEQ ID NO: 18 - protein, 120 aa, synthetic construct
  REGION 1..120: note = synthetic
EVQLVESGGGLVQPGGSLRLSCAASGFTFSSYVMSWVRQAPGKGLEWVSAIIGSGGSTYYADSVKGRFTISRDNSKNTLYLQMNSLRAEDTAVYYCAKRAGDNWNWFDPWGQGTLVTVSS

SEQ ID NO: 19 - DNA, 24 bp, synthetic construct
  misc_feature 1..24: note = synthetic
  source 1..24: mol_type = other DNA
ggattcacctttagcagctatgtc

SEQ ID NO: 20 - protein, 8 aa, synthetic construct
  REGION 1..8: note = synthetic
GFTFSSYV

SEQ ID NO: 21 - DNA, 24 bp, synthetic construct
  misc_feature 1..24: note = synthetic
  source 1..24: mol_type = other DNA
attattggtagtggtggtagcaca

SEQ ID NO: 22 - protein, 8 aa, synthetic construct
  REGION 1..8: note = synthetic
IIGSGGST

SEQ ID NO: 23 - DNA, 39 bp, synthetic construct
  misc_feature 1..39: note = synthetic
  source 1..39: mol_type = other DNA
gcgaaaagagccggggataactggaactggttcgacccc

SEQ ID NO: 24 - protein, 13 aa, synthetic construct
  REGION 1..13: note = synthetic
AKRAGDNWNWFDP

SEQ ID NO: 25 - DNA, 321 bp, synthetic construct
  misc_feature 1..321: note = synthetic
  source 1..321: mol_type = other DNA
gacatccagatgacccagtctccatcttccgtgtctgcatctttaggagacagagtcaccatcacttgtcgggcgagtcagggtattagcagctggttagcctggtatcagcggaaaccagggaaagcccctaagctcctgatctatgctgcatccagtttgcaaagtggggtcccatcaaggttcagcggcagtggatctggggcggatttcactctcaccatcagcagcctgcagcctgaagattttgcaacttactattgtcaacaggctaaaagtgtcccattcactttcggccctgggaccaaagtggatatcaaa

SEQ ID NO: 26 - protein, 107 aa, synthetic construct
  REGION 1..107: note = synthetic
DIQMTQSPSSVSASLGDRVTITCRASQGISSWLAWYQRKPGKAPKLLIYAASSLQSGVPSRFSGSGSGADFTLTISSLQPEDFATYYCQQAKSVPFTFGPGTKVDIK

SEQ ID NO: 27 - DNA, 18 bp, synthetic construct
  misc_feature 1..18: note = synthetic
  source 1..18: mol_type = other DNA
cagggtattagcagctgg

SEQ ID NO: 28 - protein, 6 aa, synthetic construct
  REGION 1..6: note = synthetic
QGISSW

SEQ ID NO: 29-30 - skipped (2 entries)

SEQ ID NO: 31 - DNA, 27 bp, synthetic construct
  misc_feature 1..27: note = synthetic
  source 1..27: mol_type = other DNA
caacaggctaaaagtgtcccattcact

SEQ ID NO: 32 - protein, 9 aa, synthetic construct
  REGION 1..9: note = synthetic
QQAKSVPFT

SEQ ID NO: 33 - DNA, 351 bp, synthetic construct
  misc_feature 1..351: note = synthetic
  source 1..351: mol_type = other DNA
gaagtgcagctggtggagtctgggggaggcttggtacagcctggcaggtccctgagactctcctgtgcagcctctggattcacctttgatgattatgccatgcactgggtccggcaagctccagggaagggcctggagtgggtctcaggtatcagttggaatagtggtaacatgggatatgcggactctgtgaagggccgattcaccatctccagagacaacgccaagaactccctgttcctgcaaatgcacagtttgagagctgaggacacggccttttattactgtgcaaaagtccgtctaactgcctttgacttttggggccagggaaccctggtcaccgtctcctca

SEQ ID NO: 34 - protein, 117 aa, synthetic construct
  REGION 1..117: note = synthetic
EVQLVESGGGLVQPGRSLRLSCAASGFTFDDYAMHWVRQAPGKGLEWVSGISWNSGNMGYADSVKGRFTISRDNAKNSLFLQMHSLRAEDTAFYYCAKVRLTAFDFWGQGTLVTVSS

SEQ ID NO: 35 - DNA, 24 bp, synthetic construct
  misc_feature 1..24: note = synthetic
  source 1..24: mol_type = other DNA
ggattcacctttgatgattatgcc

SEQ ID NO: 36 - protein, 8 aa, synthetic construct
  REGION 1..8: note = synthetic
GFTFDDYA

SEQ ID NO: 37 - DNA, 24 bp, synthetic construct
  misc_feature 1..24: note = synthetic
  source 1..24: mol_type = other DNA
atcagttggaatagtggtaacatg

SEQ ID NO: 38 - protein, 8 aa, synthetic construct
  REGION 1..8: note = synthetic
ISWNSGNM

SEQ ID NO: 39 - DNA, 30 bp, synthetic construct
  misc_feature 1..30: note = synthetic
  source 1..30: mol_type = other DNA
gcaaaagtccgtctaactgcctttgacttt

SEQ ID NO: 40 - protein, 10 aa, synthetic construct
  REGION 1..10: note = synthetic
AKVRLTAFDF

SEQ ID NO: 41 - DNA, 321 bp, synthetic construct
  misc_feature 1..321: note = synthetic
  source 1..321: mol_type = other DNA
gacatccagatgacccagtctccatcctccctgtctgcatctgtaggagacagagtcaccatcacttgccggacaagtcagagcattggcaactatttaaattggtttcagcagaaaccagggaaagcccctaaactcctcatctatactgcatccagtttgcagaatggagtcccatcaaggttcactggcagtggatctgggacagatttcactctcaccatcagcagtctgcaacctgaggattttgtaatttactactgtcaacagagtttcagtaccccgtatacttttggccaggggaccaagctggagatcaaa

SEQ ID NO: 42 - protein, 107 aa, synthetic construct
  REGION 1..107: note = synthetic
DIQMTQSPSSLSASVGDRVTITCRTSQSIGNYLNWFQQKPGKAPKLLIYTASSLQNGVPSRFTGSGSGTDFTLTISSLQPEDFVIYYCQQSFSTPYTFGQGTKLEIK

SEQ ID NO: 43 - DNA, 18 bp, synthetic construct
  misc_feature 1..18: note = synthetic
  source 1..18: mol_type = other DNA
cagagcattggcaactat

SEQ ID NO: 44 - protein, 6 aa, synthetic construct
  REGION 1..6: note = synthetic
QSIGNY

SEQ ID NO: 45-46 - skipped (2 entries)

SEQ ID NO: 47 - DNA, 27 bp, synthetic construct
  misc_feature 1..27: note = synthetic
  source 1..27: mol_type = other DNA
caacagagtttcagtaccccgtatact

SEQ ID NO: 48 - protein, 9 aa, synthetic construct
  REGION 1..9: note = synthetic
QQSFSTPYT

SEQ ID NO: 49 - DNA, 354 bp, synthetic construct
  misc_feature 1..354: note = synthetic
  source 1..354: mol_type = other DNA
caggtgcagctggtggagtctgggggaggcttggtcaagcctggagggtccctgagactctcctgtgcagcctctggattcaccttcagtgactactacatcagctggatccgccaggctccagggaaggggctggagtgggtttcatacattagttctagtggtagttccataaagtacgcagactctgtgaagggccgattcaccatctccagggacaacgccaagaactcactgtatctgcaaatgaacagcctgagagccgaggacacggccgtatattactgtgcgagagagggagggaactacggtatggacgtctggggccaagggaccacggtcaccgtctcctca

SEQ ID NO: 50 - protein, 118 aa, synthetic construct
  REGION 1..118: note = synthetic
QVQLVESGGGLVKPGGSLRLSCAASGFTFSDYYISWIRQAPGKGLEWVSYISSSGSSIKYADSVKGRFTISRDNAKNSLYLQMNSLRAEDTAVYYCAREGGNYGMDVWGQGTTVTVSS

SEQ ID NO: 51 - DNA, 24 bp, synthetic construct
  misc_feature 1..24: note = synthetic
  source 1..24: mol_type = other DNA
ggattcaccttcagtgactactac

SEQ ID NO: 52 - protein, 8 aa, synthetic construct
  REGION 1..8: note = synthetic
GFTFSDYY

SEQ ID NO: 53 - DNA, 24 bp, synthetic construct
  misc_feature 1..24: note = synthetic
  source 1..24: mol_type = other DNA
attagttctagtggtagttccata

SEQ ID NO: 54 - protein, 8 aa, synthetic construct
  REGION 1..8: note = synthetic
ISSSGSSI

SEQ ID NO: 55 - DNA, 33 bp, synthetic construct
  misc_feature 1..33: note = synthetic
  source 1..33: mol_type = other DNA
gcgagagagggagggaactacggtatggacgtc

SEQ ID NO: 56 - protein, 11 aa, synthetic construct
  REGION 1..11: note = synthetic
AREGGNYGMDV

SEQ ID NO: 57 - DNA, 321 bp, synthetic construct
  misc_feature 1..321: note = synthetic
  source 1..321: mol_type = other DNA
gacatccagatgacccagtctccatcttccgtgtctgcatctgtaggagacagagtcaccatcacttgtcgggcgagtcagggtattaacaactggttagtctggtatcagcagaaaccagggaaagcccctaagctcctgatctatgctgcaaccagcttgcaaagtggggtcccatcaaggttcagcggcagtgggtctgggacagatttcactctcaccatcagcagcctgcagcctgaagattttgcaacttactattgtcaacaggctaacagtttccctcccacttttggccaggggaccaagctggagatcaaa

SEQ ID NO: 58 - protein, 107 aa, synthetic construct
  REGION 1..107: note = synthetic
DIQMTQSPSSVSASVGDRVTITCRASQGINNWLVWYQQKPGKAPKLLIYAATSLQSGVPSRFSGSGSGTDFTLTISSLQPEDFATYYCQQANSFPPTFGQGTKLEIK

SEQ ID NO: 59 - DNA, 18 bp, synthetic construct
  misc_feature 1..18: note = synthetic
  source 1..18: mol_type = other DNA
cagggtattaacaactgg

SEQ ID NO: 60 - protein, 6 aa, synthetic construct
  REGION 1..6: note = synthetic
QGINNW

SEQ ID NO: 61-62 - skipped (2 entries)

SEQ ID NO: 63 - DNA, 27 bp, synthetic construct
  misc_feature 1..27: note = synthetic
  source 1..27: mol_type = other DNA
caacaggctaacagtttccctcccact

SEQ ID NO: 64 - protein, 9 aa, synthetic construct
  REGION 1..9: note = synthetic
QQANSFPPT

SEQ ID NO: 65 - DNA, 375 bp, synthetic construct
  misc_feature 1..375: note = synthetic
  source 1..375: mol_type = other DNA
gaggtgcagctggtggagtctgggggaggcttggtccagcctggggggtccctgagactctcctgtgcagcctctggattcacctttagtaacttttggatgacctgggtccgccaggctccagggaaggggctggagtgggtggccaacatgaaccaagatggaagtgagaaatactatgtggactctgtgaagggccgattcaccatctccagagacaacgccaagagctcactgtatctgcaaatgaacagcctgagagccgaggacacggctgtgtattactgtgcgagagatcgggaatattgtattagtaccagctgctatgatgactttgactactggggccagggaaccctggtcaccgtctcctca

SEQ ID NO: 66 - protein, 125 aa, synthetic construct
  REGION 1..125: note = synthetic
EVQLVESGGGLVQPGGSLRLSCAASGFTFSNFWMTWVRQAPGKGLEWVANMNQDGSEKYYVDSVKGRFTISRDNAKSSLYLQMNSLRAEDTAVYYCARDREYCISTSCYDDFDYWGQGTLVTVSS

SEQ ID NO: 67 - DNA, 24 bp, synthetic construct
  misc_feature 1..24: note = synthetic
  source 1..24: mol_type = other DNA
ggattcacctttagtaacttttgg

SEQ ID NO: 68 - protein, 8 aa, synthetic construct
  REGION 1..8: note = synthetic
GFTFSNFW

SEQ ID NO: 69 - DNA, 24 bp, synthetic construct
  misc_feature 1..24: note = synthetic
  source 1..24: mol_type = other DNA
atgaaccaagatggaagtgagaaa

SEQ ID NO: 70 - protein, 8 aa, synthetic construct
  REGION 1..8: note = synthetic
MNQDGSEK

SEQ ID NO: 71 - DNA, 54 bp, synthetic construct
  misc_feature 1..54: note = synthetic
  source 1..54: mol_type = other DNA
gcgagagatcgggaatattgtattagtaccagctgctatgatgactttgactac

SEQ ID NO: 72 - protein, 18 aa, synthetic construct
  REGION 1..18: note = synthetic
ARDREYCISTSCYDDFDY

SEQ ID NO: 73 - DNA, 324 bp, synthetic construct
  misc_feature 1..324: note = synthetic
  source 1..324: mol_type = other DNA
gacatccagatgacccagtctccatcctccctgtctgcatctgtaggagacagagtcaccatcacttgccgggcaagtcagagcattagcagctatttaaattggtatcagcagaaaccagggaaagcccctaagctcctgatctatgctgcatccagtttgcatagtggggtcccatcaaggttcagtggcagtggatctgggacagatttcactctcaccatcagcagtctgcaacctgaagattttgcaacttactactgtcaacagagttacagtacccctccgatcaccttcggccaagggacacgactggagattaaa

SEQ ID NO: 74 - protein, 108 aa, synthetic construct
  REGION 1..108: note = synthetic
DIQMTQSPSSLSASVGDRVTITCRASQSISSYLNWYQQKPGKAPKLLIYAASSLHSGVPSRFSGSGSGTDFTLTISSLQPEDFATYYCQQSYSTPPITFGQGTRLEIK

SEQ ID NO: 75 - DNA, 18 bp, synthetic construct
  misc_feature 1..18: note = synthetic
  source 1..18: mol_type = other DNA
cagagcattagcagctat

SEQ ID NO: 76 - protein, 6 aa, synthetic construct
  REGION 1..6: note = synthetic
QSISSY

SEQ ID NO: 77-78 - skipped (2 entries)

SEQ ID NO: 79 - DNA, 30 bp, synthetic construct
  misc_feature 1..30: note = synthetic
  source 1..30: mol_type = other DNA
caacagagttacagtacccctccgatcacc

SEQ ID NO: 80 - protein, 10 aa, synthetic construct
  REGION 1..10: note = synthetic
QQSYSTPPIT

SEQ ID NO: 81 - DNA, 324 bp, synthetic construct
  misc_feature 1..324: note = synthetic
  source 1..324: mol_type = other DNA
gacatccagatgacccagtctccatcctccctgtctgcatctgtaggagacagagtcaccatcacttgccgggcaagtcagagcattagcagctatttaaattggtatcagcagaaaccagggaaagcccctaagctcctgatctatgctgcatccagtttgcaaagtggggtcccgtcaaggttcagtggcagtggatctgggacagatttcactctcaccatcagcagtctgcaacctgaagattttgcaacttactactgtcaacagagttacagtacccctccgatcaccttcggccaagggacacgactggagattaaa

SEQ ID NO: 82 - protein, 108 aa, synthetic construct
  REGION 1..108: note = synthetic
DIQMTQSPSSLSASVGDRVTITCRASQSISSYLNWYQQKPGKAPKLLIYAASSLQSGVPSRFSGSGSGTDFTLTISSLQPEDFATYYCQQSYSTPPITFGQGTRLEIK

SEQ ID NO: 83 - DNA, 18 bp, synthetic construct
  misc_feature 1..18: note = synthetic
  source 1..18: mol_type = other DNA
cagagcattagcagctat

SEQ ID NO: 84 - protein, 6 aa, synthetic construct
  REGION 1..6: note = synthetic
QSISSY

SEQ ID NO: 85-86 - skipped (2 entries)

SEQ ID NO: 87 - DNA, 30 bp, synthetic construct; identical to SEQ ID NO: 79
  misc_feature 1..30: note = synthetic
  source 1..30: mol_type = other DNA

SEQ ID NO: 88 - protein, 10 aa, synthetic construct
  REGION 1..10: note = synthetic
QQSYSTPPIT

SEQ ID NO: 89 - DNA, 372 bp, synthetic construct
  misc_feature 1..372: note = synthetic
  source 1..372: mol_type = other DNA
gaagtacagcttgtagaatccggcggaggactggtacaacctggaagaagtcttagactgagttgcgcagctagtgggtttacattcgacgattacagcatgcattgggtgaggcaagctcctggtaaaggattggaatgggttagcgggatatcatggaactcaggaagcaagggatacgccgacagcgtgaaaggccgatttacaatatctagggacaacgcaaaaaactctctctaccttcaaatgaactctcttagggcagaagacacagcattgtattattgcgcaaaatacggcagtggttatggcaagttttatcattatggactggacgtgtggggacaagggacaacagtgacagtgagtagc

SEQ ID NO: 90 - protein, 124 aa, synthetic construct
  REGION 1..124: note = synthetic
EVQLVESGGGLVQPGRSLRLSCAASGFTFDDYSMHWVRQAPGKGLEWVSGISWNSGSKGYADSVKGRFTISRDNAKNSLYLQMNSLRAEDTALYYCAKYGSGYGKFYHYGLDVWGQGTTVTVSS

SEQ ID NO: 91 - DNA, 24 bp, synthetic construct
  misc_feature 1..24: note = synthetic
  source 1..24: mol_type = other DNA
gggtttacattcgacgattacagc

SEQ ID NO: 92 - protein, 8 aa, synthetic construct
  REGION 1..8: note = synthetic
GFTFDDYS

SEQ ID NO: 93 - DNA, 24 bp, synthetic construct
  misc_feature 1..24: note = synthetic
  source 1..24: mol_type = other DNA
atatcatggaactcaggaagcaag

SEQ ID NO: 94 - protein, 8 aa, synthetic construct
  REGION 1..8: note = synthetic
ISWNSGSK

SEQ ID NO: 95 - DNA, 51 bp, synthetic construct
  misc_feature 1..51: note = synthetic
  source 1..51: mol_type = other DNA
gcaaaatacggcagtggttatggcaagttttatcattatggactggacgtg

SEQ ID NO: 96 - protein, 17 aa, synthetic construct
  REGION 1..17: note = synthetic
AKYGSGYGKFYHYGLDV

SEQ ID NO: 97 - DNA, 372 bp, synthetic construct
  misc_feature 1..372: note = synthetic
  source 1..372: mol_type = other DNA
gaagtacagcttgtagaatccggcggaggactggtacaacctggaagaagtcttagactgagttgcgcagctagtgggtttacattcgacgattacagcatgcattgggtgaggcaagctcctggtaaaggattggaatgggttagcgggatatcatggaactcaggaagcatcggatacgccgacagcgtgaaaggccgatttacaatatctagggacaacgcaaaaaactctctctaccttcaaatgaactctcttagggcagaagacacagcattgtattattgcgcaaaatacggcagtggttatggcaagttttattattatggaatggacgtgtggggacaagggacaacagtgacagtgagtagc

SEQ ID NO: 98 - protein, 124 aa, synthetic construct
  REGION 1..124: note = synthetic
EVQLVESGGGLVQPGRSLRLSCAASGFTFDDYSMHWVRQAPGKGLEWVSGISWNSGSIGYADSVKGRFTISRDNAKNSLYLQMNSLRAEDTALYYCAKYGSGYGKFYYYGMDVWGQGTTVTVSS

SEQ ID NO: 99 - DNA, 24 bp, synthetic construct
  misc_feature 1..24: note = synthetic
  source 1..24: mol_type = other DNA
gggtttacattcgacgattacagc

SEQ ID NO: 100 - protein, 8 aa, synthetic construct
  REGION 1..8: note = synthetic
GFTFDDYS

SEQ ID NO: 101 - DNA, 24 bp, synthetic construct
  misc_feature 1..24: note = synthetic
  source 1..24: mol_type = other DNA
atatcatggaactcaggaagcatc

SEQ ID NO: 102 - protein, 8 aa, synthetic construct
  REGION 1..8: note = synthetic
ISWNSGSI

SEQ ID NO: 103 - DNA, 51 bp, synthetic construct
  misc_feature 1..51: note = synthetic
  source 1..51: mol_type = other DNA
gcaaaatacggcagtggttatggcaagttttattattatggaatggacgtg

SEQ ID NO: 104 - protein, 17 aa, synthetic construct
  REGION 1..17: note = synthetic
AKYGSGYGKFYYYGMDV

SEQ ID NO: 105 - DNA, 249 bp, synthetic construct
  misc_feature 1..249: note = hBCMA ecto.mmh
  source 1..249: mol_type = other DNA
atgttgcagatggctgggcagtgctcccaaaatgaatattttgacagtttgttgcatgcttgcataccttgtcaacttcgatgttcttctaatactcctcctctaacatgtcagcgttattgtaatgcaagtgtgaccaattcagtgaaaggaacgaatgcggaacaaaaactcatctcagaagaggatctgggtggagaacaaaaactcatctcagaagaggatctgcaccatcaccatcaccattga

SEQ ID NO: 106 - protein, 82 aa, synthetic construct
  REGION 1..82: note = hBCMA ecto.mmh
MLQMAGQCSQNEYFDSLLHACIPCQLRCSSNTPPLTCQRYCNASVTNSVKGTNAEQKLISEEDLGGEQKLISEEDLHHHHHH

SEQ ID NO: 107 - DNA, 864 bp, synthetic construct
  misc_feature 1..864: note = hBCMA ecto.mFc
  source 1..864: mol_type = other DNA
atgttgcagatggctgggcagtgctcccaaaatgaatattttgacagtttgttgcatgcttgcataccttgtcaacttcgatgttcttctaatactcctcctctaacatgtcagcgttattgtaatgcaagtgtgaccaattcagtgaaaggaacgaatgcggagcccagagggcccacaatcaagccctgtcctccatgcaaatgcccagcacctaacctcttgggtggaccatccgtcttcatcttccctccaaagatcaaggatgtactcatgatctccctgagccccatagtcacatgtgtggtggtggatgtgagcgaggatgacccagatgtccagatcagctggtttgtgaacaacgtggaagtacacacagctcagacacaaacccatagagaggattacaacagtactctccgggtggtcagtgccctccccatccagcaccaggactggatgagtggcaaggagttcaaatgcaaggtcaacaacaaagacctcccagcgcccatcgagagaaccatctcaaaacccaaagggtcagtaagagctccacaggtatatgtcttgcctccaccagaagaagagatgactaagaaacaggtcactctgacctgcatggtcacagacttcatgcctgaagacatttacgtggagtggaccaacaacgggaaaacagagctaaactacaagaacactgaaccagtcctggactctgatggttcttacttcatgtacagcaagctgagagtggaaaagaagaactgggtggaaagaaatagctactcctgttcagtggtccacgagggtctgcacaatcaccacacgactaagagcttctcccggactccgggtaaatga

SEQ ID NO: 108 - protein, 287 aa, synthetic construct
  REGION 1..287: note = hBCMA ecto.mFc
MLQMAGQCSQNEYFDSLLHACIPCQLRCSSNTPPLTCQRYCNASVTNSVKGTNAEPRGPTIKPCPPCKCPAPNLLGGPSVFIFPPKIKDVLMISLSPIVTCVVVDVSEDDPDVQISWFVNNVEVHTAQTQTHREDYNSTLRVVSALPIQHQDWMSGKEFKCKVNNKDLPAPIERTISKPKGSVRAPQVYVLPPPEEEMTKKQVTLTCMVTDFMPEDIYVEWTNNGKTELNYKNTEPVLDSDGSYFMYSKLRVEKKNWVERNSYSCSVVHEGLHNHHTTKSFSRTPGK

SEQ ID NO: 109 - DNA, 246 bp, synthetic construct
  misc_feature 1..246: note = mfBCMA ecto.mmh
  source 1..246: mol_type = other DNA
atgttgcagatggctcggcagtgctcccaaaatgaatattttgacagtttgttgcatgattgcaaaccttgtcaacttcgatgttctagtactcctcctctaacatgtcagcgttattgcaatgcaagtatgaccaattcagtgaaaggaatgaatgcggaacaaaaactcatctcagaagaggatctgggtggagaacaaaaactcatctcagaagaggatctgcaccatcaccatcaccattga

SEQ ID NO: 110 - protein, 81 aa, synthetic construct
  REGION 1..81: note = mfBCMA ecto.mmh
MLQMARQCSQNEYFDSLLHDCKPCQLRCSSTPPLTCQRYCNASMTNSVKGMNAEQKLISEEDLGGEQKLISEEDLHHHHHH

SEQ ID NO: 111 - DNA, 861 bp, synthetic construct
  misc_feature 1..861: note = mfBCMA ecto.mFc
  source 1..861: mol_type = other DNA
atgttgcagatggctcggcagtgctcccaaaatgaatattttgacagtttgttgcatgattgcaaaccttgtcaacttcgatgttctagtactcctcctctaacatgtcagcgttattgcaatgcaagtatgaccaattcagtgaaaggaatgaatgcggagcccagagggcccacaatcaagccctgtcctccatgcaaatgcccagcacctaacctcttgggtggaccatccgtcttcatcttccctccaaagatcaaggatgtactcatgatctccctgagccccatagtcacatgtgtggtggtggatgtgagcgaggatgacccagatgtccagatcagctggtttgtgaacaacgtggaagtacacacagctcagacacaaacccatagagaggattacaacagtactctccgggtggtcagtgccctccccatccagcaccaggactggatgagtggcaaggagttcaaatgcaaggtcaacaacaaagacctcccagcgcccatcgagagaaccatctcaaaacccaaagggtcagtaagagctccacaggtatatgtcttgcctccaccagaagaagagatgactaagaaacaggtcactctgacctgcatggtcacagacttcatgcctgaagacatttacgtggagtggaccaacaacgggaaaacagagctaaactacaagaacactgaaccagtcctggactctgatggttcttacttcatgtacagcaagctgagagtggaaaagaagaactgggtggaaagaaatagctactcctgttcagtggtccacgagggtctgcacaatcaccacacgactaagagcttctcccggactccgggtaaatga

SEQ ID NO: 112 - protein, 286 aa, synthetic construct
  REGION 1..286: note = mfBCMA ecto.mFc
MLQMARQCSQNEYFDSLLHDCKPCQLRCSSTPPLTCQRYCNASMTNSVKGMNAEPRGPTIKPCPPCKCPAPNLLGGPSVFIFPPKIKDVLMISLSPIVTCVVVDVSEDDPDVQISWFVNNVEVHTAQTQTHREDYNSTLRVVSALPIQHQDWMSGKEFKCKVNNKDLPAPIERTISKPKGSVRAPQVYVLPPPEEEMTKKQVTLTCMVTDFMPEDIYVEWTNNGKTELNYKNTEPVLDSDGSYFMYSKLRVEKKNWVERNSYSCSVVHEGLHNHHTTKSFSRTPGK

SEQ ID NO: 113 - DNA, 849 bp, synthetic construct
  misc_feature 1..849: note = Mouse BCMA ecto domain with mouse Fc
  source 1..849: mol_type = other DNA
atggcgcaacagtgtttccacagtgaatattttgacagtctgctgcatgcttgcaaaccgtgtcacttgcgatgttccaaccctcctgcaacctgtcagccttactgtgatccaagcgtgaccagttcagtgaaagggacgtacacggagcccagagggcccacaatcaagccctgtcctccatgcaaatgcccagcacctaacctcttgggtggaccatccgtcttcatcttccctccaaagatcaaggatgtactcatgatctccctgagccccatagtcacatgtgtggtggtggatgtgagcgaggatgacccagatgtccagatcagctggtttgtgaacaacgtggaagtacacacagctcagacacaaacccatagagaggattacaacagtactctccgggtggtcagtgccctccccatccagcaccaggactggatgagtggcaaggagttcaaatgcaaggtcaacaacaaagacctcccagcgcccatcgagagaaccatctcaaaacccaaagggtcagtaagagctccacaggtatatgtcttgcctccaccagaagaagagatgactaagaaacaggtcactctgacctgcatggtcacagacttcatgcctgaagacatttacgtggagtggaccaacaacgggaaaacagagctaaactacaagaacactgaaccagtcctggactctgatggttcttacttcatgtacagcaagctgagagtggaaaagaagaactgggtggaaagaaatagctactcctgttcagtggtccacgagggtctgcacaatcaccacacgactaagagcttctcccggactccgggtaaatga

SEQ ID NO: 114 - protein, 282 aa, synthetic construct
  REGION 1..282: note = Mouse BCMA ecto domain with mouse Fc
MAQQCFHSEYFDSLLHACKPCHLRCSNPPATCQPYCDPSVTSSVKGTYTEPRGPTIKPCPPCKCPAPNLLGGPSVFIFPPKIKDVLMISLSPIVTCVVVDVSEDDPDVQISWFVNNVEVHTAQTQTHREDYNSTLRVVSALPIQHQDWMSGKEFKCKVNNKDLPAPIERTISKPKGSVRAPQVYVLPPPEEEMTKKQVTLTCMVTDFMPEDIYVEWTNNGKTELNYKNTEPVLDSDGSYFMYSKLRVEKKNWVERNSYSCSVVHEGLHNHHTTKSFSRTPGK

SEQ ID NO: 115 - protein, 184 aa, synthetic construct
  REGION 1..184: note = human BCMA (TNFRSF17) Protein NP_001183.2
MLQMAGQCSQNEYFDSLLHACIPCQLRCSSNTPPLTCQRYCNASVTNSVKGTNAILWTCLGLSLIISLAVFVLMFLLRKINSEPLKDEFKNTGSGLLGMANIDLEKSRTGDEIILPRGLEYTVEECTCEDCIKSKPKVDSDHCFPLPAMEEGATILVTTKTNDYCKSLPAALSATEIEKSISAR

SEQ ID NO: 116 - protein, 207 aa, synthetic construct
  REGION 1..207: note = human CD3 Epsilon Protein (>NP_000724.1 T-cell surface glycoprotein CD3 epsilon chain precursor
MQSGTHWRVLGLCLLSVGVWGQDGNEEMGGITQTPYKVSISGTTVILTCPQYPGSEILWQHNDKNIGGDEDDKNIGSDEDHLSLKEFSELEQSGYYVCYPRGSKPEDANFYLYLRARVCENCMEMDVMSVATIVIVDICITGGLLLLVYYWSKNRKAKAKPVTRGAGAGGRQRGQNKERPPPVPNPDYEPIRKGQRDLYSGLNQRRI

SEQ ID NO: 117 - protein, 171 aa, synthetic construct
  REGION 1..171: note = human CD3 Delta Protein (>NP_000723.1 T-cell surface glycoprotein CD3 delta chain isoform A precursor
MEHSTFLSGLVLATLLSQVSPFKIPIEELEDRVFVNCNTSITWVEGTVGTLLSDITRLDLGKRILDPRGIYRCNGTDIYKDKESTVQVHYRMCQSCVELDPATVAGIIVTDVIATLLLALGVFCFAGHETGRLSGAADTQALLRNDQVYQPLRDRDDAQYSHLGGNWARNK

SEQ ID NO: 118 - protein, 164 aa, synthetic construct
  REGION 1..164: note = human CD3 Zeta Protein (>NP_932170.1 T-cell surface glycoprotein CD3 zeta chain isoform 1 precursor
MKWKALFTAAILQAQLPITEAQSFGLLDPKLCYLLDGILFIYGVILTALFLRVKFSRSADAPAYQQGQNQLYNELNLGRREEYDVLDKRRGRDPEMGGKPQRRKNPQEGLYNELQKDKMAEAYSEIGMKGERRRGKGHDGLYQGLSTATKDTYDALHMQALPPR

SEQ ID NO: 119 - protein, 182 aa, synthetic construct
  REGION 1..182: note = human CD3 Gamma Protein (>NP_000064.1 T-cell surface glycoprotein CD3 gamma chain precursor
MEQGKGLAVLILAIILLQGTLAQSIKGNHLVKVYDYQEDGSVLLTCDAEAKNITWFKDGKMIGFLTEDKKKWNLGSNAKDPRGMYQCKGSQNKSKPLQVYYRMCQNCIELNAATISGFLFAEIVSIFVLAVGVYFIAGQDGVRQSRASDKQTLLPNDQLYQPLKDREDDQYSHLQGNQLRRN

SEQ ID NO: 120 - protein, 281 aa, synthetic construct
  REGION 1..281: note = Human BCMA ecto.hFc Protein
MLQMAGQCSQNEYFDSLLHACIPCQLRCSSNTPPLTCQRYCNASVTNSVKGTNADKTHTCPPCPAPELLGGPSVFLFPPKPKDTLMISRTPEVTCVVVDVSHEDPEVKFNWYVDGVEVHNAKTKPREEQYNSTYRVVSVLTVLHQDWLNGKEYKCKVSNKALPAPIEKTISKAKGQPREPQVYTLPPSRDELTKNQVSLTCLVKGFYPSDIAVEWESNGQPENNYKTTPPVLDSDGSFFLYSKLTVDKSRWQQGNVFSCSVMHEALHNHYTQKSLSLSPGK

SEQ ID NO: 121 - protein, 43 aa, synthetic construct
  REGION 1..43: note = Peptides 1-43 of human BCMA
MLQMAGQCSQNEYFDSLLHACIPCQLRCSSNTPPLTCQRYCNA

SEQ ID NO: 122 - protein, 125 aa, synthetic construct
  REGION 1..125: note = 21587N VH
QVQLQESGPGLVKPSETLSLTCTVSGGSINYYYWNWIRQPPGKGLEWIGYISYSGNTNYNPSLKSRVTISVATSRNQFSLTLSSVTAADTAVYYCARFAEYCGGNICYYYGMDVWGQGTTVTVSS

SEQ ID NO: 123 - protein, 108 aa, synthetic construct
  REGION 1..108: note = 21587N VL (Non-germline Cys in CDR3)
EIVLTQSPGTLSLSPGERATFSCRASQSVGSSFLAWYQQKPGQAPRRLMYGASNRATGIPDRFSGSGSGTDFTLTISRLEPEDFAVYYCQQCGGSPWTFGQGTKVEIK

SEQ ID NO: 124 - protein, 127 aa, synthetic construct
  REGION 1..127: note = 21589N VH
QVQLVQSGAEVKRPGSSVKVSCKASGGTFSTYAINWVRQAPGQGLEWMGGIIPIFGTTNYAQKFQGRVTITTDGSTTTTYMELSSLRSEDTAVYYCARTVYDLNSKGYYYYYGLDVWGQGTTVTVSS

SEQ ID NO: 125 - protein, 114 aa, synthetic construct
  REGION 1..114: note = 21589N VL
DIVMTQTPLSLPVTPGEPASISCRSSQSLLDSDDGNTYLDWYLQKPGQSPQLLIYTLSYRASGVPDRFSGSGSGTDFTLKISRVEAEDVGIYYCMQRIEFPSLTFGGGTKVEIK